European Patent Specification EP 3 811 961 B1, published August 20, 2025. Title: STABLE POLYPEPTIDES BINDING TO HUMAN COMPLEMENT C5. Applicant: Swedish Orphan Biovitrum AB. The sequence listing filed with the application follows.

SEQUENCE LISTING (287 sequences)

SEQ ID NO: 1 - protein, 29 aa, Artificial Sequence
  Modified bacterial sequence
EVLEAWDEIDRLPNLTIEQWLAFINKLDD

SEQ ID NO: 2 - protein, 29 aa, Artificial Sequence
  Modified bacterial sequence
EVLEAWNEIDRLPNLTIEQWLAFINKLDD

SEQ ID NO: 3 - protein, 29 aa, Artificial Sequence
  Modified bacterial sequence
EVIEAWNEIDRLPNLTIEQWLAFINKLDD

SEQ ID NO: 4 - protein, 29 aa, Artificial Sequence
  Modified bacterial sequence
EVLEAWDEIDRLPNLTLDQWLAFINKLDD

SEQ ID NO: 5 - protein, 29 aa, Artificial Sequence
  Modified bacterial sequence
EVLDAWDEIDALPNLTLEQWLAFINKLDD

SEQ ID NO: 6 - protein, 29 aa, Artificial Sequence
  Modified bacterial sequence
EVIDAWDEIDRLPNLTLDQWLAFINKLDD

SEQ ID NO: 7 - protein, 29 aa, Artificial Sequence
  Modified bacterial sequence
ETLEAWDEIDRLPNLTIEQWLAFINKLDD

SEQ ID NO: 8 - protein, 29 aa, Artificial Sequence
  Modified bacterial sequence
EVIDAWNEIDALPNLTLDQWLAFINKLDD

SEQ ID NO: 9 - protein, 29 aa, Artificial Sequence
  Modified bacterial sequence
EVLDAWDEIDKLPNLTIDQWLAFINKLDD

SEQ ID NO: 10 - protein, 29 aa, Artificial Sequence
  Modified bacterial sequence
EVLEAWDEIDHLPNLTLDQWLAFINKLDD

SEQ ID NO: 11 - protein, 29 aa, Artificial Sequence
  Modified bacterial sequence
EVLEAWDEIDALPNLTIEQWLAFINKLDD

SEQ ID NO: 12 - protein, 29 aa, Artificial Sequence
  Modified bacterial sequence
EVLDAWDEIDKLPNLTLEQWLAFINKLDD

SEQ ID NO: 13 - protein, 29 aa, Artificial Sequence
  Modified bacterial sequence
ETITAWDEIDKLPNLTIEQWLAFIGKLED

SEQ ID NO: 14 - protein, 29 aa, Artificial Sequence
  Modified bacterial sequence
ESMKAWDEIDRLPNLNINQWVAFIDSLYD

SEQ ID NO: 15 - protein, 29 aa, Artificial Sequence
  Modified bacterial sequence
ESIEAWTEIDHLPNLTIEQWLAFINKLTD

SEQ ID NO: 16 - protein, 29 aa, Artificial Sequence
  Modified bacterial sequence
EVLDAWHEIDTLPNLTVRQWLAFISKLED

SEQ ID NO: 17 - protein, 29 aa, Artificial Sequence
  Modified bacterial sequence
EHIQANEEIDRLPNLTIKQWLAFINKLHD

SEQ ID NO: 18 - protein, 29 aa, Artificial Sequence
  Modified bacterial sequence
EVLHAWAEIDALPNLTIEQWLAFINKLDD

SEQ ID NO: 19 - protein, 29 aa, Artificial Sequence
  Modified bacterial sequence
EVLAAWDEIDSLPNLTLQQWLAFINKLDD

SEQ ID NO: 20 - protein, 29 aa, Artificial Sequence
  Modified bacterial sequence
EVIDAWNEIDALPNLTLEQWLAFINKLDD

SEQ ID NO: 21 - protein, 29 aa, Artificial Sequence
  Modified bacterial sequence
EVLDAWNEIDALPNLTIDQWLAFINKLSD

SEQ ID NO: 22 - protein, 29 aa, Artificial Sequence
  Modified bacterial sequence
EVIEAWDEIDGLPNLTIEQWLAFINKLDD

SEQ ID NO: 23 - protein, 29 aa, Artificial Sequence
  Modified bacterial sequence
EVLEAWDEIDHLPNLTLQQWLAFINKLDD

SEQ ID NO: 24 - protein, 29 aa, Artificial Sequence
  Modified bacterial sequence
EVIEAWNEIDALPNLTIEQWLAFINKLDD

SEQ ID NO: 25 - protein, 29 aa, Artificial Sequence
  Modified bacterial sequence
EVIAAWNEIDRLPNLTLTQWLAFINKLDD

SEQ ID NO: 26 - protein, 29 aa, Artificial Sequence
  Modified bacterial sequence
EVIEAWDEIDALPNLTLQQWLAFINKLDD

SEQ ID NO: 27 - protein, 29 aa, Artificial Sequence
  Modified bacterial sequence
EVIAAWDEIDKLPNLTIEQWLAFINKLDD

SEQ ID NO: 28 - protein, 29 aa, Artificial Sequence
  Modified bacterial sequence
EVIAAWDEIDKLPNLTLQQWLAFINKLDD

SEQ ID NO: 29 - protein, 29 aa, Artificial Sequence
  Modified bacterial sequence
ETIAAWDEIDKLPNLTIEQWLAFINKLDD

SEQ ID NO: 30 - protein, 29 aa, Artificial Sequence
  Modified bacterial sequence
ETIEAWNEIDRLPNLTIEQWLAFINKLDD

SEQ ID NO: 31 - protein, 29 aa, Artificial Sequence
  Modified bacterial sequence
EVLEAWREIDALPNLTIQQWLAFINKLDD

SEQ ID NO: 32 - protein, 29 aa, Artificial Sequence
  Modified bacterial sequence
EVIEAWDEIDQLPNLTIEQWLAFINKLDD

SEQ ID NO: 33 - protein, 29 aa, Artificial Sequence
  Modified bacterial sequence
EVLRAWDEIDHLPNLTLEQWLAFINKLDD

SEQ ID NO: 34 - protein, 29 aa, Artificial Sequence
  Modified bacterial sequence
EVLEAWDEIDRLPNLTLNQWLAFINKLDD

SEQ ID NO: 35 - protein, 29 aa, Artificial Sequence
  Modified bacterial sequence
EVLDAWNEIDHLPNLTIEQWLAFINKLDD

SEQ ID NO: 36 - protein, 29 aa, Artificial Sequence
  Modified bacterial sequence
EVIDAWNEIDKLPNLTIEQWLAFINKLDD

SEQ ID NO: 37 - protein, 29 aa, Artificial Sequence
  Modified bacterial sequence
ETLEAWDEIDQLPNLTLQQWLAFINKLDD

SEQ ID NO: 38 - protein, 29 aa, Artificial Sequence
  Modified bacterial sequence
EVIEAWNEIDALPNLTLDQWLAFINKLDD

SEQ ID NO: 39 - protein, 29 aa, Artificial Sequence
  Modified bacterial sequence
EVIDAWNEIDRLPNLTLQQWLAFINKLDD

SEQ ID NO: 40 - protein, 29 aa, Artificial Sequence
  Modified bacterial sequence
EVIDAWNEIDQLPNLTLEQWLAFINKLDD

SEQ ID NO: 41 - protein, 29 aa, Artificial Sequence
  Modified bacterial sequence
ETIAAWDEIDHLPNLTLEQWLAFINKLDD

SEQ ID NO: 42 - protein, 29 aa, Artificial Sequence
  Modified bacterial sequence
EVLQAWDEIDHLPNLTIQQWLAFINKLSD

SEQ ID NO: 43 - protein, 29 aa, Artificial Sequence
  Modified bacterial sequence
ETLHAWAEIDRLPNLTIEQWLAFINKLDD

SEQ ID NO: 44 - protein, 29 aa, Artificial Sequence
  Modified bacterial sequence
EVLEAWNEIDHLPNLTLAQWLAFINKLDD

SEQ ID NO: 45 - protein, 29 aa, Artificial Sequence
  Modified bacterial sequence
EVIEAWDEIDKLPNLTIAQWLAFINKLDD

SEQ ID NO: 46 - protein, 29 aa, Artificial Sequence
  Modified bacterial sequence
EVLDAWDEIDHLPNLTLQQWLAFINKLDD

SEQ ID NO: 47 - protein, 29 aa, Artificial Sequence
  Modified bacterial sequence
ETIEAWNEIDKLPNLTLTQWLAFINKLDD

SEQ ID NO: 48 - protein, 29 aa, Artificial Sequence
  Modified bacterial sequence
EVLEAWNEIDLLPNLTIEQWLAFINKLDD

SEQ ID NO: 49 - protein, 29 aa, Artificial Sequence
  Modified bacterial sequence
EVIEAWDEIDHLPNLTIDQWLAFINKLDD

SEQ ID NO: 50 - protein, 29 aa, Artificial Sequence
  Modified bacterial sequence
EVISAWNEIDALPNLTLQQWLAFINKLDD

SEQ ID NO: 51 - protein, 29 aa, Artificial Sequence
  Modified bacterial sequence
EVIAAWNEIDKLPNLTLEQWLAFINKLDD

SEQ ID NO: 52 - protein, 29 aa, Artificial Sequence
  Modified bacterial sequence
ETIEAWNEIDSLPNLTLDQWLAFINKLDD

SEQ ID NO: 53 - protein, 29 aa, Artificial Sequence
  Modified bacterial sequence
EVLDAWNEIDQLPNLTLQQWLAFINKLDD

SEQ ID NO: 54 - protein, 29 aa, Artificial Sequence
  Modified bacterial sequence
EVLAAWNEIDHLPNLTIEQWLAFINKLDD

SEQ ID NO: 55 - protein, 29 aa, Artificial Sequence
  Modified bacterial sequence
EVLEAWDEIDHLPNLTITQWLAFINKLDD

SEQ ID NO: 56 - protein, 29 aa, Artificial Sequence
  Modified bacterial sequence
ETIDAWNEIDHLPNLTIEQWLAFINKLDD

SEQ ID NO: 57 - protein, 29 aa, Artificial Sequence
  Modified bacterial sequence
EVIEAWNEIDHLPNLTIQQWLAFINKLDD

SEQ ID NO: 58 - protein, 29 aa, Artificial Sequence
  Modified bacterial sequence
EVIQAWNEIDALPNLTISQWLAFINKLDD

SEQ ID NO: 59 - protein, 29 aa, Artificial Sequence
  Modified bacterial sequence
EVIAAWDEIDSLPNLTIEQWLAFINKLDD

SEQ ID NO: 60 - protein, 29 aa, Artificial Sequence
  Modified bacterial sequence
EHIEAWNEIDALPNLTIEQWLAFINKLQD

SEQ ID NO: 61 - protein, 29 aa, Artificial Sequence
  Modified bacterial sequence
EVLEAWNEIDKLPNLTLDQWLAFINKLDD

SEQ ID NO: 62 - protein, 29 aa, Artificial Sequence
  Modified bacterial sequence
EVIDAWNEIDHLPNLTIEQWLAFINKLAD

SEQ ID NO: 63 - protein, 29 aa, Artificial Sequence
  Modified bacterial sequence
ETIDAWDEIDKLPNLTIEQWLAFINKLDD

SEQ ID NO: 64 - protein, 29 aa, Artificial Sequence
  Modified bacterial sequence
EVIAAWDEIDLLPNLTLQQWLAFINKLAD

SEQ ID NO: 65 - protein, 29 aa, Artificial Sequence
  Modified bacterial sequence
EVIHAWDEIDKLPNLTIEQWLAFINKLDD

SEQ ID NO: 66 - protein, 29 aa, Artificial Sequence
  Modified bacterial sequence
EVIAAWNEIDHLPNLTLEQWLAFINKLDD

SEQ ID NO: 67 - protein, 29 aa, Artificial Sequence
  Modified bacterial sequence
ETLDAWNEIDKLPNLTLSQWLAFINKLDD

SEQ ID NO: 68 - protein, 29 aa, Artificial Sequence
  Modified bacterial sequence
EVLEAWNEIDALPNLTLEQWLAFINKLDD

SEQ ID NO: 69 - protein, 29 aa, Artificial Sequence
  Modified bacterial sequence
EVIQAWDEIDHLPNLTISQWLAFINKLDD

SEQ ID NO: 70 - protein, 29 aa, Artificial Sequence
  Modified bacterial sequence
EVLQAWDEIDSLPNLTIEQWLAFINKLDD

SEQ ID NO: 71 - protein, 29 aa, Artificial Sequence
  Modified bacterial sequence
ETLEAWDEIDHLPNLTIAQWLAFINKLDD

SEQ ID NO: 72 - protein, 29 aa, Artificial Sequence
  Modified bacterial sequence
ETIDAWNEIDRLPNLTISQWLAFINKLDD

SEQ ID NO: 73 - protein, 29 aa, Artificial Sequence
  Modified bacterial sequence
EVLDAWHEIDHLPNLTIQQWLAFINKLDD

SEQ ID NO: 74 - protein, 29 aa, Artificial Sequence
  Modified bacterial sequence
EQIRAWDEIDKLPNLTIEQWLAFINKLAD

SEQ ID NO: 75 - protein, 29 aa, Artificial Sequence
  Modified bacterial sequence
ETLYAWNEIDKLPNLTIEQWLAFIEKLQD

SEQ ID NO: 76 - protein, 29 aa, Artificial Sequence
  Modified bacterial sequence
EVIEAWNEIDALPNLTIDQWLAFINKLDD

SEQ ID NO: 77 - protein, 29 aa, Artificial Sequence
  Modified bacterial sequence
EVLEAWNEIDHLPNLTIQQWLAFINKLDD

SEQ ID NO: 78 - protein, 29 aa, Artificial Sequence
  Modified bacterial sequence
ETIEAWDEIDALPNLTIEQWLAFINKLDD

SEQ ID NO: 79 - protein, 29 aa, Artificial Sequence
  Modified bacterial sequence
EVIEAWNEIDHLPNLTLQQWLAFINKLDD

SEQ ID NO: 80 - protein, 29 aa, Artificial Sequence
  Modified bacterial sequence
EVIEAWNEIDKLPNLTIQQWLAFINKLDD

SEQ ID NO: 81 - protein, 29 aa, Artificial Sequence
  Modified bacterial sequence
ETLDAWAEIDHLPNLTLDQWLAFINKLDD

SEQ ID NO: 82 - protein, 29 aa, Artificial Sequence
  Modified bacterial sequence
EHIDAWNEIDALPNLTLSQWLAFINKLDD

SEQ ID NO: 83 - protein, 29 aa, Artificial Sequence
  Modified bacterial sequence
EVLDAWNEIDKLPNLTIAQWLAFINKLDD

SEQ ID NO: 84 - protein, 29 aa, Artificial Sequence
  Modified bacterial sequence
EVIEAWTEIDYLPNLTLQQWLAFINKLDD

SEQ ID NO: 85 - protein, 29 aa, Artificial Sequence
  Modified bacterial sequence
ETIEAWNEIDHLPNLTIAQWLAFINKLDD

SEQ ID NO: 86 - protein, 29 aa, Artificial Sequence
  Modified bacterial sequence
EVIQAWNEIDKLPNLTLEQWLAFINKLDD

SEQ ID NO: 87 - protein, 29 aa, Artificial Sequence
  Modified bacterial sequence
EVIEAWDEIDHLPNLTIEQWLAFINKLDD

SEQ ID NO: 88 - protein, 29 aa, Artificial Sequence
  Modified bacterial sequence
ETIDAWNEIDLLPNLTIEQWLAFINKLDD

SEQ ID NO: 89 - protein, 29 aa, Artificial Sequence
  Modified bacterial sequence
EHIDAWNEIDKLPNLTLDQWLAFINKLDD

SEQ ID NO: 90 - protein, 29 aa, Artificial Sequence
  Modified bacterial sequence
EVVAAWNEIDALPNLTIEQWLAFINKLND

SEQ ID NO: 91 - protein, 29 aa, Artificial Sequence
  Modified bacterial sequence
EVIEAWNEIDALPNLTLAQWLAFINKLDD

SEQ ID NO: 92 - protein, 29 aa, Artificial Sequence
  Modified bacterial sequence
EVLQAWDEIDRLPNLTLDQWLAFINKLDD

SEQ ID NO: 93 - protein, 29 aa, Artificial Sequence
  Modified bacterial sequence
EVIDAWDEIDHLPNLTIEQWLAFINKLSD

SEQ ID NO: 94 - protein, 29 aa, Artificial Sequence
  Modified bacterial sequence
EVVEAWNEIDQLPNLTIEQWLAFINKLDD

SEQ ID NO: 95 - protein, 29 aa, Artificial Sequence
  Modified bacterial sequence
EVIQAWNEIDALPNLTIEQWLAFINKLDD

SEQ ID NO: 96 - protein, 29 aa, Artificial Sequence
  Modified bacterial sequence
EVIQAWDEIDKLPNLTIDQWLAFINKLAD

SEQ ID NO: 97 - protein, 29 aa, Artificial Sequence
  Modified bacterial sequence
EVVAAWDEIDALPNLTLTQWLAFINKLDD

SEQ ID NO: 98 - protein, 29 aa, Artificial Sequence
  Modified bacterial sequence
EVIQAWNEIDGLPNLTLSQWLAFINKLDD

SEQ ID NO: 99 - protein, 29 aa, Artificial Sequence
  Modified bacterial sequence
ETIEAWDEIDALPNLTITQWLAFINKLDD

SEQ ID NO: 100 - protein, 29 aa, Artificial Sequence
  Modified bacterial sequence
EVIDAWNEIDHLPNLTIQQWLAFINKLAD

SEQ ID NO: 101 - protein, 29 aa, Artificial Sequence
  Modified bacterial sequence
ETIEAWNEIDALPNLTLDQWLAFINKLED

SEQ ID NO: 102 - protein, 29 aa, Artificial Sequence
  Modified bacterial sequence
EHIHAWNEIDELPNLTIEQWLAFINKLAD

SEQ ID NO: 103 - protein, 29 aa, Artificial Sequence
  Modified bacterial sequence
EVIDAWDEIDHLPNLTIDQWLAFINKLSD

SEQ ID NO: 104 - protein, 29 aa, Artificial Sequence
  Modified bacterial sequence
EVIDANDEIDALPNLTIAQWLAFINKLHD

SEQ ID NO: 105 - protein, 29 aa, Artificial Sequence
  Modified bacterial sequence
ETIEAWDEIDKLPNLTIEQWLAFINKLDD

SEQ ID NO: 106 - protein, 29 aa, Artificial Sequence
  Modified bacterial sequence
EVLLAWDEIDHLPNLTLEQWLAFINKLDD

SEQ ID NO: 107 - protein, 29 aa, Artificial Sequence
  Modified bacterial sequence
EHIDAWNEIDGLPNLTLEQWLAFINKLDD

SEQ ID NO: 108 - protein, 29 aa, Artificial Sequence
  Modified bacterial sequence
EVIEAWSEIDALPNLTIDQWLAFINKLAD

SEQ ID NO: 109 - protein, 29 aa, Artificial Sequence
  Modified bacterial sequence
EQLNAWAEIDALPNLTIEQWLAFINKLDD

SEQ ID NO: 110 - protein, 29 aa, Artificial Sequence
  Modified bacterial sequence
EVIDAWNEIDALPNLTIAQWLAFINKLDD

SEQ ID NO: 111 - protein, 29 aa, Artificial Sequence
  Modified bacterial sequence
ETIDAWNEIDQLPNLTIEQWLAFINKLDD

SEQ ID NO: 112 - protein, 29 aa, Artificial Sequence
  Modified bacterial sequence
EVIEAWDEIDKLPNLTLAQWLAFINKLDD

SEQ ID NO: 113 - protein, 29 aa, Artificial Sequence
  Modified bacterial sequence
EVLYAWAEIDHLPNLTIEQWLAFINKLDD

SEQ ID NO: 114 - protein, 29 aa, Artificial Sequence
  Modified bacterial sequence
EQIDAWNEIDRLPNLTIQQWLAFINKLDD

SEQ ID NO: 115 - protein, 29 aa, Artificial Sequence
  Modified bacterial sequence
EVLAAWDEIDRLPNLTIEQWLAFINKLDD

SEQ ID NO: 116 - protein, 29 aa, Artificial Sequence
  Modified bacterial sequence
EVIEAWDEIDHLPNLTLHQWLAFINKLDD

SEQ ID NO: 117 - protein, 29 aa, Artificial Sequence
  Modified bacterial sequence
EVIEAWNEIDKLPNLTLQQWLAFINKLDD

SEQ ID NO: 118 - protein, 29 aa, Artificial Sequence
  Modified bacterial sequence
EVIDANDEIDALPNLTIEQWLAFINKLHD

SEQ ID NO: 119 - protein, 29 aa, Artificial Sequence
  Modified bacterial sequence
EVIAAWDEIDALPNLTIEQWLAFINKLDD

SEQ ID NO: 120 - protein, 29 aa, Artificial Sequence
  Modified bacterial sequence
EVIEAWTEIDQLPNLTLDQWLAFINKLDD

SEQ ID NO: 121 - protein, 29 aa, Artificial Sequence
  Modified bacterial sequence
EVINAWNEIDALPNLTLQQWLAFINKLDD

SEQ ID NO: 122 - protein, 29 aa, Artificial Sequence
  Modified bacterial sequence
EHIEAWDEIDHLPNLTIDQWLAFINKLAD

SEQ ID NO: 123 - protein, 29 aa, Artificial Sequence
  Modified bacterial sequence
EHLEAWREIDALPNLTIEQWLAFINKLDD

SEQ ID NO: 124 - protein, 29 aa, Artificial Sequence
  Modified bacterial sequence
EVLDAWNEIDKLPNLTLQQWLAFINKLDD

SEQ ID NO: 125 - protein, 29 aa, Artificial Sequence
  Modified bacterial sequence
EVIAAWDEIDHLPNLTIQQWLAFINKLDD

SEQ ID NO: 126 - protein, 29 aa, Artificial Sequence
  Modified bacterial sequence
EVIQAWNEIDALPNLTLEQWLAFINKLDD

SEQ ID NO: 127 - protein, 29 aa, Artificial Sequence
  Modified bacterial sequence
EVIDAWNEIDHLPNLTIAQWLAFINKLDD

SEQ ID NO: 128 - protein, 29 aa, Artificial Sequence
  Modified bacterial sequence
EQLDAWDEIDHLPNLTIDQWLAFINKLSD

SEQ ID NO: 129 - protein, 29 aa, Artificial Sequence
  Modified bacterial sequence
EVLNAWDEIDKLPNLTIEQWLAFINKLDD

SEQ ID NO: 130 - protein, 29 aa, Artificial Sequence
  Modified bacterial sequence
EVLEAWNEIDHLPNLTIDQWLAFINKLDD

SEQ ID NO: 131 - protein, 29 aa, Artificial Sequence
  Modified bacterial sequence
EVLLAWDEIDRLPNLTIDQWLAFINKLAD

SEQ ID NO: 132 - protein, 29 aa, Artificial Sequence
  Modified bacterial sequence
EVIAAWNEIDQLPNLTLDQWLAFINKLDD

SEQ ID NO: 133 - protein, 29 aa, Artificial Sequence
  Modified bacterial sequence
ETLLAWDEIDALPNLTIEQWLAFINKLDD

SEQ ID NO: 134 - protein, 29 aa, Artificial Sequence
  Modified bacterial sequence
EVIDAWNEIDTLPNLTLEQWLAFINKLDD

SEQ ID NO: 135 - protein, 29 aa, Artificial Sequence
  Modified bacterial sequence
EVLHAWNEIDHLPNLTLNQWLAFINKLQD

SEQ ID NO: 136 - protein, 29 aa, Artificial Sequence
  Modified bacterial sequence
EVIQAWNEIDALPNLTIAQWLAFINKLDD

SEQ ID NO: 137 - protein, 29 aa, Artificial Sequence
  Modified bacterial sequence
ETVDAWNEIDALPNLTIEQWLAFINKLDD

SEQ ID NO: 138 - protein, 29 aa, Artificial Sequence
  Modified bacterial sequence
EVIQAWDEIDHLPNLTIDQWLAFINKLDD

SEQ ID NO: 139 - protein, 29 aa, Artificial Sequence
  Modified bacterial sequence
EVLDAWNEIDQLPNLTIQQWLAFINKLDD

SEQ ID NO: 140 - protein, 29 aa, Artificial Sequence
  Modified bacterial sequence
ETIEAWNEIDALPNLTLDQWLAFINKLDD

SEQ ID NO: 141 - protein, 29 aa, Artificial Sequence
  Modified bacterial sequence
EVIEAWDEIDALPNLTIDQWLAFINKLDD

SEQ ID NO: 142 - protein, 29 aa, Artificial Sequence
  Modified bacterial sequence
EVIEAWNEIDQLPNLTIQQWLAFINKLDD

SEQ ID NO: 143 - protein, 29 aa, Artificial Sequence
  Modified bacterial sequence
EVIEAWTEIDHLPNLTIEQWLAFINKLDD

SEQ ID NO: 144 - protein, 29 aa, Artificial Sequence
  Modified bacterial sequence
EVIQAWNEIDHLPNLTLQQWLAFINKLED

SEQ ID NO: 145 - protein, 29 aa, Artificial Sequence
  Modified bacterial sequence
EVIQANNEIDQLPNLTIEQWLAFINKLHD

SEQ ID NO: 146 - protein, 29 aa, Artificial Sequence
  Modified bacterial sequence
EVLHAWSEIDKLPNLTIEQWLAFINKLDD

SEQ ID NO: 147 - protein, 29 aa, Artificial Sequence
  Modified bacterial sequence
ETIQAWDEIDKLPNLTLDQWLAFINKLSD

SEQ ID NO: 148 - protein, 29 aa, Artificial Sequence
  Modified bacterial sequence
ETLRAWDEIDKLPNLTIQQWLAFINKLAD

SEQ ID NO: 149 - protein, 29 aa, Artificial Sequence
  Modified bacterial sequence
EVIDAWNEIDHLPNLTIEQWLAFINKLED

SEQ ID NO: 150 - protein, 29 aa, Artificial Sequence
  Modified bacterial sequence
EVIDAWNEIDHLPNLTLQQWLAFINKLAD

SEQ ID NO: 151 - protein, 29 aa, Artificial Sequence
  Modified bacterial sequence
ETIDAWNEIDALPNLTLDQWLAFINKLDD

SEQ ID NO: 152 - protein, 29 aa, Artificial Sequence
  Modified bacterial sequence
EVIEAWNEIDQLPNLTIEQWLAFINKLDD

SEQ ID NO: 153 - protein, 29 aa, Artificial Sequence
  Modified bacterial sequence
EVIRAWDEIDQLPNLTLSQWLAFINKLDD

SEQ ID NO: 154 - protein, 29 aa, Artificial Sequence
  Modified bacterial sequence
EVIEAWNEIDRLPNLTIHQWLAFINKLDD

SEQ ID NO: 155 - protein, 29 aa, Artificial Sequence
  Modified bacterial sequence
ETIEAWNEIDQLPNLTIEQWLAFINKLDD

SEQ ID NO: 156 - protein, 29 aa, Artificial Sequence
  Modified bacterial sequence
EVLTAWAEIDALPNLTLSQWLAFINKLDD

SEQ ID NO: 157 - protein, 29 aa, Artificial Sequence
  Modified bacterial sequence
EVIEAWDEIDKLPNLTVDQWLAFINKLDD

SEQ ID NO: 158 - protein, 29 aa, Artificial Sequence
  Modified bacterial sequence
EVIDAWNEIDHLPNLTLTQWLAFINKLDD

SEQ ID NO: 159 - protein, 29 aa, Artificial Sequence
  Modified bacterial sequence
EVIEAWNEIDQLPNLTLDQWLAFINKLDD

SEQ ID NO: 160 - protein, 29 aa, Artificial Sequence
  Modified bacterial sequence
ETLQAWDEIDHLPNLTLNQWLAFINKLDD

SEQ ID NO: 161 - protein, 29 aa, Artificial Sequence
  Modified bacterial sequence
EVIDAWNEIDHLPNLTIEQWLAFINKLDD

SEQ ID NO: 162 - protein, 29 aa, Artificial Sequence
  Modified bacterial sequence
EVIEAWNEIDLLPNLTLSQWLAFINKLDD

SEQ ID NO: 163 - protein, 29 aa, Artificial Sequence
  Modified bacterial sequence
EVIDAWDEIDRLPNLTLKQWLAFINKLDD

SEQ ID NO: 164 - protein, 29 aa, Artificial Sequence
  Modified bacterial sequence
ETLHAWDEIDKLPNLTIEQWLAFINKLDD

SEQ ID NO: 165 - protein, 29 aa, Artificial Sequence
  Modified bacterial sequence
EVIKAWDEIDHLPNLTLNQWLAFINKLDD

SEQ ID NO: 166 - protein, 29 aa, Artificial Sequence
  Modified bacterial sequence
EVIEAWNEIDHLPNLTLAQWLAFINKLDD

SEQ ID NO: 167 - protein, 29 aa, Artificial Sequence
  Modified bacterial sequence
EVIQAWNEIDHLPNLTIDQWLAFITKLED

SEQ ID NO: 168 - protein, 29 aa, Artificial Sequence
  Modified bacterial sequence
EVIEAWNEIDRLPNLTIKQWLAFINKLDD

SEQ ID NO: 169 - protein, 29 aa, Artificial Sequence
  Modified bacterial sequence
EVIEAWNEIDSLPNLTLQQWLAFINKLDD

SEQ ID NO: 170 - protein, 29 aa, Artificial Sequence
  Modified bacterial sequence
ETIDAWNEIDKLPNLTIEQWLAFINKLDD

SEQ ID NO: 171 - protein, 29 aa, Artificial Sequence
  Modified bacterial sequence
EVLEAWAEIDALPNLTIAQWLAFINKLDD

SEQ ID NO: 172 - protein, 29 aa, Artificial Sequence
  Modified bacterial sequence
ETIDAWNEIDRLPNLTIEQWLAFINKLDD

SEQ ID NO: 173 - protein, 29 aa, Artificial Sequence
  Modified bacterial sequence
ETLKAWDEIDRLPNLTLEQWLAFINKLDD

SEQ ID NO: 174 - protein, 29 aa, Artificial Sequence
  Modified bacterial sequence
ETIAAWNEIDALPNLTLQQWLAFINKLDD

SEQ ID NO: 175 - protein, 29 aa, Artificial Sequence
  Modified bacterial sequence
EVLQAWNEIDHLPNLTIQQWLAFINKLDD

SEQ ID NO: 176 - protein, 29 aa, Artificial Sequence
  Modified bacterial sequence
EVIEAWSEIDHLPNLTLQQWLAFINKLDD

SEQ ID NO: 177 - protein, 29 aa, Artificial Sequence
  Modified bacterial sequence
EVIDAWNEIDGLPNLTIEQWLAFINKLDD

SEQ ID NO: 178 - protein, 29 aa, Artificial Sequence
  Modified bacterial sequence
EVIHAWNEIDHLPNLTLNQWLAFINKLED

SEQ ID NO: 179 - protein, 29 aa, Artificial Sequence
  Modified bacterial sequence
EVLDAWNEIDSLPNLTLDQWLAFINKLDD

SEQ ID NO: 180 - protein, 29 aa, Artificial Sequence
  Modified bacterial sequence
EQIEAWNEIDRLPNLTLEQWLAFINKLDD

SEQ ID NO: 181 - protein, 29 aa, Artificial Sequence
  Modified bacterial sequence
EVVDAWNEIDALPNLTLQQWLAFINKLDD

SEQ ID NO: 182 - protein, 29 aa, Artificial Sequence
  Modified bacterial sequence
EVIEAWNEIDKLPNLTIEQWLAFINKLDD

SEQ ID NO: 183 - protein, 29 aa, Artificial Sequence
  Modified bacterial sequence
EVIEANDEIDRLPNLTIEQWLAFINKLHD

SEQ ID NO: 184 - protein, 29 aa, Artificial Sequence
  Modified bacterial sequence
ETLQAWDEIDKLPNLTIEQWLAFINKLDD

SEQ ID NO: 185 - protein, 29 aa, Artificial Sequence
  Modified bacterial sequence
EVIEAWDEIDHLPNLTIDQWLAFINKLAD

SEQ ID NO: 186 - protein, 29 aa, Artificial Sequence
  Modified bacterial sequence
ETIDAWNEIDHLPNLTLQQWLAFINKLAD

SEQ ID NO: 187 - protein, 29 aa, Artificial Sequence
  Modified bacterial sequence
EVIDAWDEIDKLPNLTIEQWLAFINKLDD

SEQ ID NO: 188 - protein, 29 aa, Artificial Sequence
  Modified bacterial sequence
EVIEAWNEIDKLPNLTLAQWLAFINKLDD

SEQ ID NO: 189 - protein, 29 aa, Artificial Sequence
  Modified bacterial sequence
EVLQAWDEIDKLPNLTIQQWLAFINKLDD

SEQ ID NO: 190 - protein, 29 aa, Artificial Sequence
  Modified bacterial sequence
EVIAAWNEIDGLPNLTLQQWLAFINKLDD

SEQ ID NO: 191 - protein, 29 aa, Artificial Sequence
  Modified bacterial sequence
ETLNAWNEIDALPNLTLQQWLAFINKLDD

SEQ ID NO: 192 - protein, 29 aa, Artificial Sequence
  Modified bacterial sequence
EVLSAWNEIDQLPNLTLEQWLAFINKLDD

SEQ ID NO: 193 - protein, 29 aa, Artificial Sequence
  Modified bacterial sequence
ETLEAWDEIDHLPNLTLHQWLAFINKLDD

SEQ ID NO: 194 - protein, 29 aa, Artificial Sequence
  Modified bacterial sequence
EQIEAWNEIDHLPNLTLQQWLAFINKLAD

SEQ ID NO: 195 - protein, 29 aa, Artificial Sequence
  Modified bacterial sequence
EVVEAWDEIDKLPNLTIEQWLAFINKLDD

SEQ ID NO: 196 - protein, 29 aa, Artificial Sequence
  Modified bacterial sequence
EVLEAWNEIDELPNLTIEQWLAFINKLDD

SEQ ID NO: 197 - protein, 29 aa, Artificial Sequence
  Modified bacterial sequence
EVIDAWNEIDQLPNLTLQQWLAFINKLDD

SEQ ID NO: 198 - protein, 29 aa, Artificial Sequence
  Modified bacterial sequence
ETIDAWDEIDKLPNLTLSQWLAFINKLDD

SEQ ID NO: 199 - protein, 29 aa, Artificial Sequence
  Modified bacterial sequence
ETIDAWNEIDQLPNLTLQQWLAFINKLDD

SEQ ID NO: 200 - protein, 29 aa, Artificial Sequence
  Modified bacterial sequence
EVIQAWDEIDALPNLTLNQWLAFINKLDD

SEQ ID NO: 201 - protein, 29 aa, Artificial Sequence
  Modified bacterial sequence
EVLDAWAEIDQLPNLTLQQWLAFINKLDD

SEQ ID NO: 202 - protein, 29 aa, Artificial Sequence
  Modified bacterial sequence
EHIAAWDEIDALPNLTIEQWLAFINKLDD

SEQ ID NO: 203 - protein, 29 aa, Artificial Sequence
  Modified bacterial sequence
EVIRAWDEIDALPNLTIEQWLAFINKLDD

SEQ ID NO: 204 - protein, 29 aa, Artificial Sequence
  Modified bacterial sequence
EVIDAWDEIDALPNLTIDQWLAFINKLAD

SEQ ID NO: 205 - protein, 29 aa, Artificial Sequence
  Modified bacterial sequence
EVIDAWNEIDRLPNLTIQQWLAFINKLDD

SEQ ID NO: 206 - protein, 29 aa, Artificial Sequence
  Modified bacterial sequence
EVITAWNEIDHLPNLTLSQWLAFINKLDD

SEQ ID NO: 207 - protein, 29 aa, Artificial Sequence
  Modified bacterial sequence
EVIDAWNEIDALPNLTIHQWLAFINKLDD

SEQ ID NO: 208 - protein, 29 aa, Artificial Sequence
  Modified bacterial sequence
EQLKAWDEIDKLPNLTIEQWLAFIEKLQD

SEQ ID NO: 209 - protein, 29 aa, Artificial Sequence
  Modified bacterial sequence
EHIDAWTEIDHLPNLTIEQWLAFINKLDD

SEQ ID NO: 210 - protein, 29 aa, Artificial Sequence
  Modified bacterial sequence
EQLRAWDEIDKLPNLTIEQWLAFINKLQD

SEQ ID NO: 211 - protein, 29 aa, Artificial Sequence
  Modified bacterial sequence
EVLEAWREIDSLPNLTIAQWLAFINKLDD

SEQ ID NO: 212 - protein, 29 aa, Artificial Sequence
  Modified bacterial sequence
EVIQAWNEIDKLPNLTIEQWLAFINKLDD

SEQ ID NO: 213 - protein, 29 aa, Artificial Sequence
  Modified bacterial sequence
EHVEAWNEIDQLPNLTIEQWLAFINKLAD

SEQ ID NO: 214 - protein, 29 aa, Artificial Sequence
  Modified bacterial sequence
EVIDAWDEIDALPNLTIDQWLAFINKLSD

SEQ ID NO: 215 - protein, 29 aa, Artificial Sequence
  Modified bacterial sequence
EVIEAWNEIDHLPNLTIEQWLAFINKLDD

SEQ ID NO: 216 - protein, 29 aa, Artificial Sequence
  Modified bacterial sequence
EVLQAWDEIDKLPNLTIEQWLAFINKLSD

SEQ ID NO: 217 - protein, 29 aa, Artificial Sequence
  Modified bacterial sequence
EVIKAWNEIDSLPNLTIEQWLAFINKLDD

SEQ ID NO: 218 - protein, 29 aa, Artificial Sequence
  Modified bacterial sequence
EVLEAWHEIDLLPNLTIQQWLAFINKLDD

SEQ ID NO: 219 - protein, 29 aa, Artificial Sequence
  Modified bacterial sequence
EVLEAWTEIDRLPNLTLDQWLAFINKLDD

SEQ ID NO: 220 - protein, 29 aa, Artificial Sequence
  Modified bacterial sequence
EQLYAWNEIDHLPNLTIEQWLAFIEKLQD

SEQ ID NO: 221 - protein, 29 aa, Artificial Sequence
  Modified bacterial sequence
EVLNAWDEIDKLPNLTIKQWLAFINKLDD

SEQ ID NO: 222 - protein, 29 aa, Artificial Sequence
  Modified bacterial sequence
EVIRAWDEIDKLPNLTVEQWLAFINKLDD

SEQ ID NO: 223 - protein, 29 aa, Artificial Sequence
  Modified bacterial sequence
EVVQAWDEIDQLPNLTLEQWLAFINKLDD

SEQ ID NO: 224 - protein, 29 aa, Artificial Sequence
  Modified bacterial sequence
EVIRAWDEIDQLPNLTLEQWLAFINKLDD

SEQ ID NO: 225 - protein, 29 aa, Artificial Sequence
  Modified bacterial sequence
ETIDAWNEIDHLPNLTLDQWLAFINKLDD

SEQ ID NO: 226 - protein, 29 aa, Artificial Sequence
  Modified bacterial sequence
EVVAAWTEIDLLPNLTLDQWLAFINKLED

SEQ ID NO: 227 - protein, 29 aa, Artificial Sequence
  Modified bacterial sequence
EVVAAWDEIDALPNLTIEQWLAFINKLSD

SEQ ID NO: 228 - protein, 29 aa, Artificial Sequence
  Modified bacterial sequence
ETLEAWREIDSLPNLTLEQWLAFINKLDD

SEQ ID NO: 229 - protein, 29 aa, Artificial Sequence
  Modified bacterial sequence
EVIKAWNEIDHLPNLTLDQWLAFINKLDD

SEQ ID NO: 230 - protein, 29 aa, Artificial Sequence
  Modified bacterial sequence
EVLEAWTEIDKLPNLTIDQWLAFINKLDD

SEQ ID NO: 231 - protein, 29 aa, Artificial Sequence
  Modified bacterial sequence
ETLEAWDEIDKLPNLTIDQWLAFINKLDD

SEQ ID NO: 232 - protein, 29 aa, Artificial Sequence
  Modified bacterial sequence
EVIEAWNEIDKLPNLTIDQWLAFINKLDD

SEQ ID NO: 233 - protein, 29 aa, Artificial Sequence
  Modified bacterial sequence
ETIDAWNEIDKLPNLTLEQWLAFINKLDD

SEQ ID NO: 234 - protein, 29 aa, Artificial Sequence
  Modified bacterial sequence
ETLDAWDEIDALPNLTIDQWLAFINKLED

SEQ ID NO: 235 - protein, 29 aa, Artificial Sequence
  Modified bacterial sequence
EVLSAWNEIDHLPNLTIQQWLAFINKLDD

SEQ ID NO: 236 - protein, 29 aa, Artificial Sequence
  Modified bacterial sequence
EVIQANDEIDKLPNLTIEQWLAFIHKLHD

SEQ ID NO: 237 - protein, 29 aa, Artificial Sequence
  Modified bacterial sequence
EHLDAWDEIDHLPNLTIQQWLAFINKLAD

SEQ ID NO: 238 - protein, 29 aa, Artificial Sequence
  Modified bacterial sequence
EVIQAWNEIDQLPNLTIEQWLAFINKLDD

SEQ ID NO: 239 - protein, 29 aa, Artificial Sequence
  Modified bacterial sequence
EVIEAWNEIDYLPNLTIAQWIAFINKLDD

SEQ ID NO: 240 - protein, 29 aa, Artificial Sequence
  Modified bacterial sequence
ETIQAWDEIDRLPNLTLQQWLAFINKLDD

SEQ ID NO: 241 - protein, 29 aa, Artificial Sequence
  Modified bacterial sequence
ETIQAWDEIDKLPNLTIEQWLAFINKLDD

SEQ ID NO: 242 - protein, 29 aa, Artificial Sequence
  Modified bacterial sequence
ETLDAWAEIDHLPNLTIEQWLAFINKLDD

SEQ ID NO: 243 - protein, 29 aa, Artificial Sequence
  Modified bacterial sequence
EVIEAWDEIDKLPNLTLNQWLAFINKLDD

SEQ ID NO: 244 - protein, 29 aa, Artificial Sequence
  Modified bacterial sequence
EVLDAWNEIDQLPNLTIEQWLAFINKLDD

SEQ ID NO: 245 - protein, 29 aa, Artificial Sequence
  Modified bacterial sequence
EVLHAWNEIDHLPNLTIEQWLAFIEKLED

SEQ ID NO: 246 - protein, 29 aa, Artificial Sequence
  Modified bacterial sequence
EVIEAWQEIDKLPNLTIDQWLAFINKLDD

SEQ ID NO: 247 - protein, 29 aa, Artificial Sequence
  Modified bacterial sequence
EVVDAWNEIDQLPNLTIEQWLAFINKLDD

SEQ ID NO: 248 - protein, 29 aa, Artificial Sequence
  Modified bacterial sequence
EQIEAWNEIDALPNLTIEQWLAFINKLAD

SEQ ID NO: 249 - protein, 108 aa, Artificial Sequence
  Modified bacterial sequence
AEAKYAKEVLEAWDEIDRLPNLTIEQWLAFINKLDDDPSQSSELLSEAKKLNDSQAPKVDGSLAEAKEAANAELDSYGVSDFYKRLIDKAKTVEGVEALKDAILAALP

SEQ ID NO: 250 - protein, 46 aa, Artificial Sequence
  Modified bacterial sequence
LAEAKEAANAELDSYGVSDFYKRLIDKAKTVEGVEALKDAILAALP

SEQ ID NO: 251 - protein, 1676 aa, Homo sapiens
MGLLGILCFLIFLGKTWGQEQTYVISAPKIFRVGASENIVIQVYGYTEAFDATISIKSYPDKKFSYSSGHVHLSSENKFQNSAILTIQPKQLPGGQNPVSYVYLEVVSKHFSKSKRMPITYDNGFLFIHTDKPVYTPDQSVKVRVYSLNDDLKPAKRETVLTFIDPEGSEVDMVEEIDHIGIISFPDFKIPSNPRYGMWTIKAKYKEDFSTTGTAYFEVKEYVLPHFSVSIEPEYNFIGYKNFKNFEITIKARYFYNKVVTEADVYITFGIREDLKDDQKEMMQTAMQNTMLINGIAQVTFDSETAVKELSYYSLEDLNNKYLYIAVTVIESTGGFSEEAEIPGIKYVLSPYKLNLVATPLFLKPGIPYPIKVQVKDSLDQLVGGVPVTLNAQTIDVNQETSDLDPSKSVTRVDDGVASFVLNLPSGVTVLEFNVKTDAPDLPEENQAREGYRAIAYSSLSQSYLYIDWTDNHKALLVGEHLNIIVTPKSPYIDKITHYNYLILSKGKIIHFGTREKFSDASYQSINIPVTQNMVPSSRLLVYYIVTGEQTAELVSDSVWLNIEEKCGNQLQVHLSPDADAYSPGQTVSLNMATGMDSWVALAAVDSAVYGVQRGAKKPLERVFQFLEKSDLGCGAGGGLNNANVFHLAGLTFLTNANADDSQENDEPCKEILRPRRTLQKKIEEIAAKYKHSVVKKCCYDGACVNNDETCEQRAARISLGPRCIKAFTECCVVASQLRANISHKDMQLGRLHMKTLLPVSKPEIRSYFPESWLWEVHLVPRRKQLQFALPDSLTTWEIQGVGISNTGICVADTVKAKVFKDVFLEMNIPYSVVRGEQIQLKGTVYNYRTSGMQFCVKMSAVEGICTSESPVIDHQGTKSSKCVRQKVEGSSSHLVTFTVLPLEIGLHNINFSLETWFGKEILVKTLRVVPEGVKRESYSGVTLDPRGIYGTISRRKEFPYRIPLDLVPKTEIKRILSVKGLLVGEILSAVLSQEGINILTHLPKGSAEAELMSVVPVFYVFHYLETGNHWNIFHSDPLIEKQKLKKKLKEGMLSIMSYRNADYSYSVWKGGSASTWLTAFALRVLGQVNKYVEQNQNSICNSLLWLVENYQLDNGSFKENSQYQPIKLQGTLPVEARENSLYLTAFTVIGIRKAFDICPLVKIDTALIKADNFLLENTLPAQSTFTLAISAYALSLGDKTHPQFRSIVSALKREALVKGNPPIYRFWKDNLQHKDSSVPNTGTARMVETTAYALLTSLNLKDINYVNPVIKWLSEEQRYGGGFYSTQDTINAIEGLTEYSLLVKQLRLSMDIDVSYKHKGALHNYKMTDKNFLGRPVEVLLNDDLIVSTGFGSGLATVHVTTVVHKTSTSEEVCSFYLKIDTQDIEASHYRGYGNSDYKRIVACASYKPSREESSSGSSHAVMDISLPTGISANEEDLKALVEGVDQLFTDYQIKDGHVILQLNSIPSSDFLCVRFRIFELFEVGFLSPATFTVYEYHRPDKQCTMFYSTSNIKIQKVCEGAACKCVEADCGQMQEELDLTISAETRKQTACKPEIAYAYKVSITSITVENVFVKYKATLLDIYKTGEAVAEKDSEITFIKKVTCTNAELVKGRQYLIMGKEALQIKYNFSFRYIYPLDSLTWIEYWPRDTTCSSCQAFLANLDEFAEDIFLNGC

SEQ ID NO: 252 - protein, 108 aa, Artificial Sequence
  Modified bacterial sequence
AEAKYAKEVLEAWDEIDRLPNLTIEQWLAFINKLDRQPEQSSELLSEAKKLNDSQAPKVDGSLAEAKEAANAELDSYGVSDFYKRLIDKAKTVEGVEALKDAILAALP

SEQ ID NO: 253 - protein, 108 aa, Artificial Sequence
  Modified bacterial sequence
AEAKYAKEVLEAWDEIDRLPNLTIEQWLAFINKLDDDPSQSSELLSEAKKLSESQAPKVDGSLAEAKEAANAELDSYGVSDFYKRLIDKAKTVEGVEALKDAILAALP

SEQ ID NO: 254 - protein, 108 aa, Artificial Sequence
  Modified bacterial sequence
AEAKYAKEVLEAWDEIDRLPNLTIEQWLAFINKLDDDPSQSSELLSEAKKLNDSQAPKVDGSLAEAKVLANRELDKYGVSDFYKRLINKAKTVEGVEALKLHILAALP

SEQ ID NO: 255 - protein, 108 aa, Artificial Sequence
  Modified bacterial sequence
AEAKYAKEVLEAWSEIDRLPNLTIEQWLAFINKLDDDPSQSSELLSEAKKLNDSQAPKVDGSLAEAKEAANAELDSYGVSDFYKRLIDKAKTVEGVEALKDAILAALP

SEQ ID NO: 256 - protein, 108 aa, Artificial Sequence
  Modified bacterial sequence
AEAKYAKEVLEAWDEIERLPNLTIEQWLAFINKLDDDPSQSSELLSEAKKLNDSQAPKVDGSLAEAKEAANAELDSYGVSDFYKRLIDKAKTVEGVEALKDAILAALP

SEQ ID NO: 257 - protein, 108 aa, Artificial Sequence
  Modified bacterial sequence
AEAKYAKEVLEAWDEIDRLPNLTIEQWLAFIAKLDDDPSQSSELLSEAKKLNDSQAPKVDGSLAEAKEAANAELDSYGVSDFYKRLIDKAKTVEGVEALKDAILAALP

SEQ ID NO: 258 - protein, 108 aa, Artificial Sequence
  Modified bacterial sequence
AEAKYAKEVLEAWDEIDRLPNLTIEQWLAFINKLEDDPSQSSELLSEAKKLNDSQAPKVDGSLAEAKEAANAELDSYGVSDFYKRLIDKAKTVEGVEALKDAILAALP

SEQ ID NO: 259 - protein, 103 aa, Artificial Sequence
  Modified bacterial sequence
AEAKYAKEVLEAWDEIDRLPNLTIEQWLAFINKLDDDPSQSSELLSEAKKLNDSQAPLAEAKEAANAELDSYGVSDFYKRLIDKAKTVEGVEALKDAILAALP

SEQ ID NO: 260 - protein, 57 aa, Artificial Sequence
  Modified bacterial sequence
AEAKYAKEVLEAWDEIDRLPNLTIEQWLAFINKLDDDPSQSSELLSEAKKLSESQAP

SEQ ID NO: 261 - protein, 108 aa, Artificial Sequence
  Modified bacterial sequence
AEAKYAKEVLEAWDEIDRLPNLTIEQWLAFINKLDDDPSQSSELLSEAKKLSESQAPKVEGSLAEAKEAANAELDSYGVSDFYKRLIDKAKTVEGVEALKDAILAALP

SEQ ID NO: 262 - protein, 108 aa, Artificial Sequence
  Modified bacterial sequence
AEAKYAKEVLEAWDEIDRLPNLTIEQWLAFINKLDDDPSQSSELLSEAKKLSESQAPKVAGSLAEAKEAANAELDSYGVSDFYKRLIDKAKTVEGVEALKDAILAALP

SEQ ID NO: 263 - protein, 108 aa, Artificial Sequence
  Modified bacterial sequence
AEAKYAKEVLEAWDEIDRLPNLTIEQWLAFINKLDDDPSQSSELLSEAKKLESSQAPKVEGSLAEAKEAANAELDSYGVSDFYKRLIDKAKTVEGVEALKDAILAALP

SEQ ID NO: 264 - protein, 108 aa, Artificial Sequence
  Modified bacterial sequence
AEAKYAKEVLEAWDEIDRLPNLTIEQWLAFINKLDRQPEQSSELLSEAKKLSESQAPKVEGSLAEAKEAANAELDSYGVSDFYKRLIDKAKTVEGVEALKDAILAALP

SEQ ID NO: 265 - protein, 57 aa, Artificial Sequence
  Modified bacterial sequence
AEAKYAKEVLEAWDEIDRLPNLTIEQWLAFINKLDDDPSQSSELLSEAKKLESSQAP

SEQ ID NO: 266 - protein, 57 aa, Artificial Sequence
  Modified bacterial sequence
AEAKYAKEVLEAWDEIDRLPNLTIEQWLAFINKLDRQPEQSSELLSEAKKLSESQAP

SEQ ID NO: 267 - protein, 58 aa, Artificial Sequence
  Modified bacterial sequence
AEAKYAKEVLEAWDEIDRLPNLTIEQWLAFINKLDDDPSQSSELLSEAKKLSESQAPK

SEQ ID NO: 268 - protein, 108 aa, Artificial Sequence
  Modified bacterial sequence
AEAKYAKEVLEAWDEIDRLPNLTIEQWLAFINKLDDDPSQSSELLSEAKKLNDSQAPKVEGSLAEAKEAANAELDSYGVSDFYKRLIDKAKTVEGVEALKDAILAALP

SEQ ID NO: 269 - protein, 108 aa, Artificial Sequence
  Modified bacterial sequence
AEAKYAKEVLEAWDEIDRLPNLTIEQWLAFINKLDDDPSQSSELLSEAKKLNESQAPKVEGSLAEAKEAANAELDSYGVSDFYKRLIDKAKTVEGVEALKDAILAALP

SEQ ID NO: 270 - protein, 108 aa, Artificial Sequence
  Modified bacterial sequence
AEAKYAKEVLEAWDEIDRLPNLTIEQWLAFINKLDDDPSQSSELLSEAKKLSDSQAPKVEGSLAEAKEAANAELDSYGVSDFYKRLIDKAKTVEGVEALKDAILAALP

SEQ ID NO: 271 - protein, 62 aa, Artificial Sequence
  Modified bacterial sequence
AEAKYAKEVLEAWDEIDRLPNLTIEQWLAFINKLDDDPSQSSELLSEAKKLNDSQAPKVDGS

SEQ ID NO: 272 - protein, 58 aa, Artificial Sequence
  Modified bacterial sequence
AEAKYAKEMRNAYWEIALLPNLTNQQKRAFIRKLYDDPSQSSELLSEAKKLNDSQAPK

SEQ ID NO: 273 - protein, 58 aa, Artificial Sequence
  Modified bacterial sequence
AEAKYAKEMRNAYWEIALLPNLTNQQKRAFIRKLYDDPSQSSELLSEAKKLSESQAPK

SEQ ID NO: 274 - protein, 58 aa, Artificial Sequence
  Modified bacterial sequence
AEAKYAKEMRNAYWEIALLPNLTNQQKRAFIRKLYRQPEQSSELLSEAKKLSESQAPK

SEQ ID NO: 275 - protein, 58 aa, Artificial Sequence
  Modified bacterial sequence
AEAKYAKELIEAAAEIDALPNLTRRQWNAFIKKLVDDPSQSSELLSEAKKLNDSQAPK

SEQ ID NO: 276 - protein, 58 aa, Artificial Sequence
  Modified bacterial sequence
AEAKYAKELIEAAAEIDALPNLTRRQWNAFIKKLVDDPSQSSELLSEAKKLSESQAPK

SEQ ID NO: 277 - protein, 58 aa, Artificial Sequence
  Modified bacterial sequence
AEAKYAKELIEAAAEIDALPNLTRRQWNAFIKKLVRQPEQSSELLSEAKKLSESQAPK

SEQ ID NO: 278 - protein, 58 aa, Artificial Sequence
  Modified bacterial sequence
AEAKYAKEQDAAAHEIRWLPNLTFDQRVAFIHKLADDPSQSSELLSEAKKLNDSQAPK

SEQ ID NO: 279 - protein, 58 aa, Artificial Sequence
  Modified bacterial sequence
AEAKYAKEQDAAAHEIRWLPNLTFDQRVAFIHKLADDPSQSSELLSEAKKLSESQAPK

SEQ ID NO: 280 - protein, 58 aa, Artificial Sequence
  Modified bacterial sequence
AEAKYAKEQDAAAHEIRWLPNLTFDQRVAFIHKLARQPEQSSELLSEAKKLSESQAPK

SEQ ID NO: 281 - protein, 58 aa, Artificial Sequence
  Modified bacterial sequence
AEAKYAKENLFAGWEISDLPNLTDYQRNAFIYKLWDDPSQSSELLSEAKKLNDSQAPK

SEQ ID NO: 282 - protein, 58 aa, Artificial Sequence
  Modified bacterial sequence
AEAKYAKENLFAGWEISDLPNLTDYQRNAFIYKLWDDPSQSSELLSEAKKLSESQAPK

SEQ ID NO: 283 - protein, 58 aa, Artificial Sequence
  Modified bacterial sequence
AEAKYAKENLFAGWEISDLPNLTDYQRNAFIYKLWRQPEQSSELLSEAKKLSESQAPK

SEQ ID NO: 284 - protein, 58 aa, Artificial Sequence
  Modified bacterial sequence
AEAKYAKENLFAGWEISDLPNLTDYQRNAFIYKLWDDPSQSSELLSEAKKLNESQAPK

SEQ ID NO: 285 - protein, 58 aa, Artificial Sequence
  Modified bacterial sequence
AEAKYAKENLFAGWEISDLPNLTDYQRNAFIYKLWRQPEQSSELLSEAKKLNESQAPK

SEQ ID NO: 286 - protein, 58 aa, Artificial Sequence
  Modified bacterial sequence
AEAKYAKENLFAGWEISDLPNLTDYQRNAFIYKLWDDPSQSSELLSEAKKLSDSQAPK

SEQ ID NO: 287 - protein, 58 aa, Artificial Sequence
  Modified bacterial sequence
AEAKYAKENLFAGWEISDLPNLTDYQRNAFIYKLWRQPEQSSELLSEAKKLSDSQAPK